European Patent Specification EP 4 073 270 B1, published January 21, 2026. Title: RAPID AMPLIFICATION AND GENOTYPING OF NUCLEIC ACID SEQUENCES. Applicant: Belak, Sandor Granberg, Fredrik. The sequence listing filed with the application follows.

SEQUENCE LISTING (48 sequences)

SEQ ID NO: 1 - DNA, 24 bp, Artificial Sequence
  amplification primer
ttcaatcattcaaatctcaacttt

SEQ ID NO: 2 - DNA, 24 bp, Artificial Sequence
  amplification primer
caatttcatcattcattcatttca

SEQ ID NO: 3 - DNA, 24 bp, Artificial Sequence
  reverse primer
tcatttcaatcaatcatcaacaat

SEQ ID NO: 4 - DNA, 18 bp, Artificial Sequence
  probe for RPE-labelling
caatttcatcattcattc

SEQ ID NO: 5 - DNA, 44 bp, Artificial Sequence
  selection primer
ttcaatcattcaaatctcaactttcgttgctggccgtrcatttg

SEQ ID NO: 6 - DNA, 68 bp, Artificial Sequence
  barcoding primer
caatttcatcattcattcatttcattcacttttcaatcaactttaatccatttgtacggctccgcagt

SEQ ID NO: 7 - DNA, 44 bp, Artificial Sequence
  selection primer
tcatttcaatcaatcatcaacaatgtcattgcgctgccattctc

SEQ ID NO: 8 - DNA, 24 bp, Artificial Sequence
  capture probe
ttcacttttcaatcaactttaatc

SEQ ID NO: 9 - DNA, 44 bp, Artificial Sequence
  selection primer
ttcaatcattcaaatctcaactttagaagaagcacgcccgacac

SEQ ID NO: 10 - DNA, 56 bp, Artificial Sequence
  barcoding primer
caatttcatcattcattcatttcatacatcaacaattcattcaatacacgcaagag

SEQ ID NO: 11 - DNA, 44 bp, Artificial Sequence
  selection primer
tcatttcaatcaatcatcaacaatgcccagttgtgatgcattcg

SEQ ID NO: 12 - DNA, 24 bp, Artificial Sequence
  capture probe
tacatcaacaattcattcaataca

SEQ ID NO: 13 - DNA, 44 bp, Artificial Sequence
  selection primer
ttcaatcattcaaatctcaactttgcagactgggtgtggcattg

SEQ ID NO: 14 - DNA, 68 bp, Artificial Sequence
  barcoding primer
caatttcatcattcattcatttcaatcattacaatccaatcaattcattgcgatgtgcagcaccagta

SEQ ID NO: 15 - DNA, 44 bp, Artificial Sequence
  selection primer
tcatttcaatcaatcatcaacaattgacgtgcttttccgcaatc

SEQ ID NO: 16 - DNA, 24 bp, Artificial Sequence
  capture probe
atcattacaatccaatcaattcat

SEQ ID NO: 17 - DNA, 44 bp, Artificial Sequence
  selection primer
ttcaatcattcaaatctcaactttsatgggwgccaatcgggtta

SEQ ID NO: 18 - DNA, 69 bp, Artificial Sequence
  barcoding primer
caatttcatcattcattcatttcacaattcaaatcacaataatcaatccaatcgggttattggcaatgg

SEQ ID NO: 19 - DNA, 43 bp, Artificial Sequence
  selection primer
tcatttcaatcaatcatcaacaataggcgtcaccctcgaaggt

SEQ ID NO: 20 - DNA, 24 bp, Artificial Sequence
  capture probe
caattcaaatcacaataatcaatc

SEQ ID NO: 21 - DNA, 44 bp, Artificial Sequence
  selection primer
ttcaatcattcaaatctcaacttttacgcatgtgcctggaggag

SEQ ID NO: 22 - DNA, 67 bp, Artificial Sequence
  barcoding primer
caatttcatcattcattcatttcaaatcaatcttcattcaaatcatcaggttccgctggatcgcaag

SEQ ID NO: 23 - DNA, 44 bp, Artificial Sequence
  selection primer
tcatttcaatcaatcatcaacaatgctcgttcggagcatgaaca

SEQ ID NO: 24 - DNA, 24 bp, Artificial Sequence
  capture probe
aatcaatcttcattcaaatcatca

SEQ ID NO: 25 - DNA, 44 bp, Artificial Sequence
  selection probe
ttcaatcattcaaatctcaactttgcctggcaactgtgaaagca

SEQ ID NO: 26 - DNA, 68 bp, Artificial Sequence
  barcoding probe
caatttcatcattcattcatttcaatacttcattcattcatcaattcacaccgcagagccacaaaatg

SEQ ID NO: 27 - DNA, 44 bp, Artificial Sequence
  selection probe
tcatttcaatcaatcatcaacaatgctgcgccctctctttggta

SEQ ID NO: 28 - DNA, 24 bp, Artificial Sequence
  capture probe
atacttcattcattcatcaattca

SEQ ID NO: 29 - DNA, 44 bp, Artificial Sequence
  selection primer
ttcaatcattcaaatctcaactttcgcccagatcctcaactgga

SEQ ID NO: 30 - DNA, 68 bp, Artificial Sequence
  barcoding primer
caatttcatcattcattcatttcaaatcctttttactcaattcaatcaggacaagatgggcggtatgg

SEQ ID NO: 31 - DNA, 44 bp, Artificial Sequence
  selection primer
tcatttcaatcaatcatcaacaatggggccggggtaaaatacct

SEQ ID NO: 32 - DNA, 24 bp, Artificial Sequence
  capture probe
aatcctttttactcaattcaatca

SEQ ID NO: 33 - DNA, 44 bp, Artificial Sequence
  selection primer
ttcaatcattcaaatctcaacttttccgatcagatgcaccgtgt

SEQ ID NO: 34 - DNA, 69 bp, Artificial Sequence
  barcoding primer
caatttcatcattcattcatttcaaatcctttctttaatctcaaatcacgacgagattgtgcggttctt

SEQ ID NO: 35 - DNA, 46 bp, Artificial Sequence
  selection primer
tcatttcaatcaatcatcaacaatacaccgagaccaatagcggaag

SEQ ID NO: 36 - DNA, 24 bp, Artificial Sequence
  capture probe
aatcctttctttaatctcaaatca

SEQ ID NO: 37 - DNA, 44 bp, Artificial Sequence
  selection primer
ttcaatcattcaaatctcaactttcgacggcrcaggctacatcc

SEQ ID NO: 38 - DNA, 68 bp, Artificial Sequence
  barcoding primer
caatttcatcattcattcatttcatacaaatcatcaatcactttaatctcccgatyatggtcctgctt

SEQ ID NO: 39 - DNA, 44 bp, Artificial Sequence
  selection primer
tcatttcaatcaatcatcaacaatcgcatagatcgccgtgaaga

SEQ ID NO: 40 - DNA, 24 bp, Artificial Sequence
  capture probe
tacaaatcatcaatcactttaatc

SEQ ID NO: 41 - DNA, 46 bp, Artificial Sequence
  selection primer
ttcaatcattcaaatctcaacttttccacaaacgctgaaattgctc

SEQ ID NO: 42 - DNA, 69 bp, Artificial Sequence
  barcoding primer
caatttcatcattcattcatttcataatcttctatatcaacatcttacacaccaaagacgtggatgcaa

SEQ ID NO: 43 - DNA, 49 bp, Artificial Sequence
  selection primer
tcatttcaatcaatcatcaacaatttaagctactttcgagccatgcttc

SEQ ID NO: 44 - DNA, 24 bp, Artificial Sequence
  capture probe
taatcttctatatcaacatcttac

SEQ ID NO: 45 - DNA, 44 bp, Artificial Sequence
  selection primer
ttcaatcattcaaatctcaactttgctcacccagaaacgctggt

SEQ ID NO: 46 - DNA, 67 bp, Artificial Sequence
  barcoding primer
aatttcatcattcattcatttcaatcaaatctcatcaattcaacaatgcatcttacggatggcatga

SEQ ID NO: 47 - DNA, 43 bp, Artificial Sequence
  selection primer
catttcaatcaatcatcaacaatttcggtcctccgatcgttgt

SEQ ID NO: 48 - DNA, 24 bp, Artificial Sequence
  capture probe
atcaaatctcatcaattcaacaat